European Patent Specification EP 4 244 346 B1, published July 8, 2026. Title: Engineered Chimeric Antimicrobial Agents against Gram-Positive Bacteria. Applicant: Massachusetts Institute of Technology. The sequence listing filed with the application follows.

SEQUENCE LISTING (20 sequences)

SEQ ID NO: 1 - DNA, 20 bp, Artificial Sequence
  PlyV12 insert forward primer
ctgaacggtggttctacccc

SEQ ID NO: 2 - DNA, 21 bp, Artificial Sequence
  PlyV12 insert reverse primer
tttgaaggtaccccacgcttc

SEQ ID NO: 3 - DNA, 47 bp, Artificial Sequence
  PlyV12 P10N-V12C forward primer
cgtccgccgtacgaaaaagataccccgctgaacggtggttctacccc

SEQ ID NO: 4 - DNA, 51 bp, Artificial Sequence
  PlyV12 P10N-V12C reverse primer
ggatcctcaatggtggtgatgatggtgcgctttgaaggtaccccacgcttc

SEQ ID NO: 5 - DNA, 16 bp, Artificial Sequence
  LysEF-P10 insert forward primer
gcgccgaaaccgccgg

SEQ ID NO: 6 - DNA, 27 bp, Artificial Sequence
  LysEF-P10 insert reverse primer
cgcaactttgaactgcgggtgagacag

SEQ ID NO: 7 - DNA, 46 bp, Artificial Sequence
  LysEF-P10 V12N-P10C forward primer
gtatagcatgggttggtacgtttatcgtctggcgccgaaaccgccg

SEQ ID NO: 8 - DNA, 53 bp, Artificial Sequence
  LysEF-P10 V12N-P10C reverse primer
ggatcctcaatggtggtgatgatggtgcgcaactttgaactgcgggtgagaca

SEQ ID NO: 9 - protein, 338 aa, Artificial Sequence
  Lysin LKCHAPV12 amino acid sequence
MAKTQAEINKRLDAYAKGTVDSPYRVKKATSYDPSFGVMEAGAIDADGYYHAQCQDLITDYVLWLTDNKVRTWGNAKDQIKQSYGTGFKIHENKPSTVPKKGWIAVFTSGSYEQWGHIGIVYDGGNTSTFTILEQNWNGYANKKPTKRVDNYYGLTHFIEIPVKAGSSGLNGGSTPPKPNTKKVKVLKHATNWSPSSKGAKMASFVKGGTFEVKQQRPISYSYSNQEYLIVNKGTVLGWVLSQDIEGGYGSDRVGGSKPKLPAGFTKEEATFINGNAPITTRKNKPSLSSQTATPLYPGQSVRYLGWKSAEGYIWIYATDGRYIPVRPVGKEAWGTFK

SEQ ID NO: 10 - DNA, 1014 bp, Artificial Sequence
  Lysin LKCHAPV12 nucleotide sequence
atggctaaaacccaggctgaaattaacaaacgtctggatgcgtacgcaaaaggtactgttgattccccgtatcgtgttaaaaaagcgaccagctacgatccgtccttcggtgttatggaagcgggtgcgatcgatgcagacggctactaccacgcacagtgtcaggatctgatcaccgattatgttctgtggctgaccgataacaaagttcgtacctggggtaacgcgaaagatcagatcaaacagtcttacggcaccggtttcaaaatccatgaaaacaaaccgagcaccgttccgaaaaaaggctggattgcggtttttacttctggctcttacgaacagtggggtcacatcggtatcgtttatgatggtggtaacaccagcaccttcaccattctggaacagaactggaacggttatgcgaacaaaaaaccgaccaaacgtgttgataactattatggtctgacccacttcattgaaatcccggttaaagcgggctcttctggtctgaacggtggtagcaccccgccgaaaccgaacaccaaaaaagttaaagttctgaaacatgcaaccaactggagcccgtctagcaaaggcgcgaaaatggcatccttcgttaaaggcggcacctttgaagttaaacagcagcgtccgatcagctactcttatagcaaccaggaatacctgatcgttaacaaaggtactgttctgggctgggttctgagccaggatattgaaggtggttacggttccgatcgtgttggtggttctaaaccgaaactgccggcgggtttcaccaaagaagaagcgaccttcattaacggtaacgcgccgatcactacccgtaaaaataaaccgagcctgagttctcagaccgcgaccccgctgtatccgggtcagtctgttcgttatctgggctggaaatctgcggaaggttacatctggatctacgcgaccgatggtcgttatatcccggttcgtccggttggtaaagaagcgtggggcaccttcaaa

SEQ ID NO: 11 - protein, 321 aa, Artificial Sequence
  Lysin P10N-V12C amino acid sequence
MVKVNDVVSYLNSRVGTGIDMDGAYGFQCADLAQAITYNFFGWWFYGNAIALASQPIPNGFERIRVTDATQIKAGDIVVWSEHEYAQYGHVAIAAKDGYSDQTFENYAQNWLNASLTVGSPIALVRTNMYGVGYVIRPPYEKDTPLNGGSTPPKPNTKKVKVLKHATNWSPSSKGAKMASFVKGGTFEVKQQRPISYSYSNQEYLIVNKGTVLGWVLSQDIEGGYGSDRVGGSKPKLPAGFTKEEATFINGNAPITTRKNKPSLSSQTAIPLYPGQSVRYLGWKSAEGYIWIYATDGRYIPVRPVGKEAWGTFKAHHHHHH

SEQ ID NO: 12 - DNA, 963 bp, Artificial Sequence
  Lysin P10N-V12C nucleotide sequence
atggttaaagttaacgatgttgttagctacctgaactctcgtgttggtaccggtatcgatatggatggtgcgtacggtttccagtgcgcggatctggcgcaggcgatcacctacaacttcttcggttggtggttctacggcaacgcgatcgcactggcgtctcagccgatcccgaacggcttcgaacgtatccgtgttaccgatgcgacccagatcaaagcgggcgatatcgttgtttggagcgaacacgaatacgcgcagtacggtcacgttgcgatcgcggcgaaagatggctacagcgatcagaccttcgaaaactacgcgcagaactggctgaacgcgagcctgaccgttggtagcccgatcgcgctggttcgtaccaacatgtacggcgttggttacgttatccgtccgccgtacgaaaaagataccccgctgaacggtggttctaccccgcctaaaccgaacactaaaaaagttaaagttctgaaacatgcaaccaactggtctccgagctctaaaggtgcgaaaatggctagcttcgttaaaggcggtactttcgaagttaaacagcagcgtccgattagctactcttactctaaccaggaatacctgattgttaacaaaggtaccgttctgggttgggttctgagccaggatattgaaggtggttacggctctgatcgtgttggcggtagcaaaccgaaactgccggctggtttcaccaaagaagaagcgaccttcatcaacggtaacgctccgatcaccacccgtaaaaacaaaccgtctctgtctagccagaccgcgatcccgctgtatccgggtcagagcgttcgttacctgggctggaaatctgctgaaggttacatctggatctacgcgaccgatggtcgttacatcccggttcgtccggttggtaaagaagcgtggggtaccttcaaagcgcaccatcatcaccaccat

SEQ ID NO: 13 - protein, 242 aa, Artificial Sequence
  Lysin V12NM3 amino acid sequence
MSNINMETAIANMYALKARGITYSMNYSRTGADGTGDCSGTVYDSLRKAGASDAGWVLNTDSMHSWLEKNGFKLIAQNKEWSAKRGDVVIFGKKGASGGSAGHVVIFISSTQIIHCTWKSATANGVYVDNEATTCPYSMGWYVYRGSSGKSASKITVGSKAPYNLKWSKGAYFNAKIDGLGATSATRYGDNRTNYRFDVGQAVYAPGTLIYVFEIIDGWCRIYWNNHNEWIWHERLIVKEVF

SEQ ID NO: 14 - DNA, 726 bp, Artificial Sequence
  Lysin V12NM3 nucleotide sequence
atgtctaacattaacatggaaaccgcgatcgctaacatgtatgctctgaaagcgcgtggtatcacctactctatgaactacagccgtaccggtgctgatggcaccggtgattgttctggcaccgtttacgattctctgcgtaaagcaggtgcttctgatgcgggttgggttctgaacaccgatagcatgcacagctggctggagaaaaacggcttcaaactgattgctcagaacaaagaatggtctgcaaaacgtggtgatgttgttatctttggtaaaaaaggtgcatctggtggcagcgcgggtcacgttgttatcttcatcagctccacccagatcattcattgcacctggaaaagcgctaccgcgaacggtgtttacgttgataacgaagctaccacctgtccgtactctatgggttggtacgtttaccgtggctcttctggtaaatctgcgagcaaaatcaccgttggttctaaagcgccgtacaacctgaaatggtctaaaggtgcgtacttcaacgcaaaaatcgatggtctgggtgcgacctctgcgacccgttacggtgataaccgtaccaactaccgtttcgatgttggtcaggcggtttacgcgccgggcaccctgatctacgttttcgaaatcatcgatggttggtgccgtatctattggaacaaccacaacgaatggatctggcacgaacgtctgatcgttaaagaagttttc

SEQ ID NO: 15 - protein, 262 aa, Artificial Sequence
  Lysin LKNM3 amino acid sequence
MAKTQAEINKRLDAYAKGTVDSPYRVKKATSYDPSFGVMEAGAIDADGYYHAQCQDLITDYVLWLTDNKVRTWGNAKDQIKQSYGTGFKIHENKPSTVPKKGWIAVFTSGSYEQWGHIGIVYDGGNTSTFTILEQNWNGYANKKPTKRVDNYYGLTHFIEIPVKAGSSGKSASKITVGSKAPYNLKWSKGAYFNAKIDGLGATSATRYGDNRTNYRFDVGQAVYAPGTLIYVFEIIDGWCRIYWNNHNEWIWHERLIVKEVF

SEQ ID NO: 16 - DNA, 786 bp, Artificial Sequence
  Lysin LKNM3 nucleotide sequence
atggctaaaacccaggctgaaattaacaaacgtctggatgcgtacgcaaaaggtactgttgattccccgtatcgtgttaaaaaagcgaccagctacgatccgtccttcggtgttatggaagcgggtgcgatcgatgcagacggctactaccacgcacagtgtcaggatctgatcaccgattatgttctgtggctgaccgataacaaagttcgtacctggggtaacgcgaaagatcagatcaaacagtcttacggcaccggtttcaaaatccatgaaaacaaaccgagcaccgttccgaaaaaaggctggattgcggtttttacttctggctcttacgaacagtggggtcacatcggtatcgtttatgatggtggtaacaccagcaccttcaccattctggaacagaactggaacggttatgcgaacaaaaaaccgaccaaacgtgttgataactattatggtctgacccacttcattgaaatcccggttaaagcgggttcttctggtaaatctgcgagcaaaatcaccgttggttctaaagcgccgtacaacctgaaatggtctaaaggtgcgtacttcaacgcaaaaatcgatggtctgggtgcgacctctgcgacccgttacggtgataaccgtaccaactaccgtttcgatgttggtcaggcggtttacgcgccgggcaccctgatctacgttttcgaaatcatcgatggttggtgccgtatctattggaacaaccacaacgaatggatctggcacgaacgtctgatcgttaaagaagttttc

SEQ ID NO: 17 - protein, 321 aa, Artificial Sequence
  Lysin PlyV12 amino acid sequence
MSNINMETAIANMYALKARGITYSMNYSRTGADGTGDCSGTVYDSLRKAGASDAGWVLNTDSMHSWLEKNGFKLIAQNKEWSAKRGDVVIFGKKGASGGSAGHVVIFISSTQIIHCTWKSATANGVYVDNEATTCPYSMGWYVYRLNGGSTPPKPNTKKVKVLKHATNWSPSSKGAKMASFVKGGTFEVKQQRPISYSYSNQEYLIVNKGTVLGWVLSQDIEGGYGSDRVGGSKPKLPAGFTKEEATFINGNAPITTRKNKPSLSSQTATPLYPGQSVRYLGWKSAEGYIWIYATDGRYIPVRPVGKEAWGTFKAHHHHHH

SEQ ID NO: 18 - DNA, 963 bp, Artificial Sequence
  Lysin PlyV12 nucleotide sequence
atgtctaacatcaacatggaaaccgcaatcgctaacatgtacgcgctgaaagctcgtggtattacctatagcatgaactatagccgtaccggtgctgatggtaccggtgattgctctggcaccgtgtacgatagcctgcgtaaagcgggcgctagcgatgctggctgggttctgaacaccgattctatgcattcctggctggaaaagaacggctttaaactgatcgcacagaacaaagaatggtctgctaaacgtggtgacgttgttattttcggtaaaaaaggtgctagcggcggtagcgctggccacgttgttatcttcatcagcagcacccagattatccactgtacctggaaatctgcgaccgcgaacggtgtttacgttgataacgaagctaccacctgcccgtatagcatgggttggtacgtttatcgtctgaacggtggttctaccccgcctaaaccgaacactaaaaaagttaaagttctgaaacatgcaaccaactggtctccgagctctaaaggtgcgaaaatggctagcttcgttaaaggcggtactttcgaagttaaacagcagcgtccgattagctactcttactctaaccaggaatacctgattgttaacaaaggtaccgttctgggttgggttctgagccaggatattgaaggtggttacggctctgatcgtgttggcggtagcaaaccgaaactgccggctggtttcaccaaagaagaagcgaccttcatcaacggtaacgctccgatcaccacccgtaaaaacaaaccgtctctgtctagccagaccgcgaccccgctgtatccgggtcagagcgttcgttacctgggctggaaatctgctgaaggttacatctggatctacgcgaccgatggtcgttacatcccggttcgtccggttggtaaagaagcgtggggtaccttcaaagcgcaccatcatcaccaccat

SEQ ID NO: 19 - protein, 260 aa, Artificial Sequence
  Lysin LysEF-P10 amino acid sequence
MHHHHHHSSGVDLGTENLYFQSMVKVNDVVSYLNSRVGTGIDMDGAYGFQCADLAQAITYNFFGWWFYGNAIALASQPIPNGFERIRVTDATQIKAGDIVVWSEHEYAQYGHVAIAAKDGYSDQTFENYAQNWLNASLTVGSPIALVRTNMYGVGYVIRPPYEKDTPAPKPPAPKPAKPNLPTPKGDDTMLAIYYKHLKNGNVEQWLLINGKRVYLPTQTWVNEANALIKAYGGTKEVVQYNHDNFGLKLLELSHPQFKV

SEQ ID NO: 20 - DNA, 780 bp, Artificial Sequence
  Lysin LysEF-P10 nucleotide sequence
atgcaccatcatcatcatcattcttctggtgtagatctgggtaccgagaacctgtacttccaatccatggttaaagttaacgatgttgttagctacctgaactctcgtgttggtaccggtatcgatatggatggtgcgtacggtttccagtgcgcggatctggcgcaggcgatcacctacaacttcttcggttggtggttctacggcaacgcgatcgcactggcgtctcagccgatcccgaacggcttcgaacgtatccgtgttaccgatgcgacccagatcaaagcgggcgatatcgttgtttggagcgaacacgaatacgcgcagtacggtcacgttgcgatcgcggcgaaagatggctacagcgatcagaccttcgaaaactacgcgcagaactggctgaacgcgagcctgaccgttggtagcccgatcgcgctggttcgtaccaacatgtacggcgttggttacgttatccgtccgccgtacgaaaaagataccccggcgccgaaaccgccggctccgaaaccggctaaaccgaacctgccgaccccgaaaggtgatgataccatgctggctatctattacaaacatctgaaaaacggtaacgttgaacagtggctgctgattaacggtaaacgcgtttacctgccgacccagacctgggttaacgaagcgaacgctctgattaaagcgtatggtggcaccaaagaagttgttcagtataaccatgataacttcggcctgaaactgctggaactgtctcacccgcagttcaaagtt